European Patent Specification EP 3 830 119 B1, published November 12, 2025. Title: Anti-BTN3A antibodies and their use in treating cancer or infectious disorders. Applicant: IMCHECK THERAPEUTICS. The sequence listing filed with the application follows.

SEQUENCE LISTING (23 sequences)

SEQ ID NO: 1 - protein, 122 aa, Homo sapiens [sequence omitted]

SEQ ID NO: 2 - protein, 107 aa, Homo sapiens
DIQMTQSPSSLSASVGDRVTITCHASQNINVWLSWYQQKPGKAPKLLIYKASNLHTGVPSRFTGSGSGTDFTFTISSLQPEDIATYYCQQGQTYPYTFGQGTKLEIK

SEQ ID NO: 3 - protein, 107 aa, Homo sapiens
DIQMTQSPSSLSASVGDRVTITCHASQNINVWLSWYQQKPGKAPKLLIYKASNLHTGVPSRFSGSGSGTDFTFTISSLQPEDIATYYCQQGQTYPYTFGQGTKLEIK

SEQ ID NO: 4 - protein, 451 aa, Homo sapiens
QVQLVQSGAEVKKPGASVKLSCKASGYIFTRYYMYWVKQRPGQGLEWIGEINPNNGGTKFNEKFKNRATLTVDKSISTAYMELSRLRSDDTAVYYCSREDDYDGTPFAMDYWGQGTLVTVSSASTKGPSVFPLAPSSKSTSGGTAALGCLVKDYFPEPVTVSWNSGALTSGVHTFPAVLQSSGLYSLSSVVTVPSSSLGTQTYICNVNHKPSNTKVDKRVEPKSCDKTHTCPPCPAPEFEGGPSVFLFPPKPKDTLMISRTPEVTCVVVDVSHEDPEVKFNWYVDGVEVHNAKTKPREEQYNSTYRVVSVLTVLHQDWLNGKEYKCKVSNKALPASIEKTISKAKGQPREPQVYTLPPSREEMTKNQVSLTCLVKGFYPSDIAVEWESNGQPENNYKTTPPVLDSDGSFFLYSKLTVDKSRWQQGNVFSCSVMHEALHNHYTQKSLSLSPG

SEQ ID NO: 5 - protein, 448 aa, Homo sapiens
QVQLVQSGAEVKKPGASVKLSCKASGYIFTRYYMYWVKQRPGQGLEWIGEINPNNGGTKFNEKFKNRATLTVDKSISTAYMELSRLRSDDTAVYYCSREDDYDGTPFAMDYWGQGTLVTVSSASTKGPSVFPLAPCSRSTSESTAALGCLVKDYFPEPVTVSWNSGALTSGVHTFPAVLQSSGLYSLSSVVTVPSSSLGTKTYTCNVDHKPSNTKVDKRVESKYGPPCPPCPAPEFEGGPSVFLFPPKPKDTLMISRTPEVTCVVVDVSQEDPEVQFNWYVDGVEVHNAKTKPREEQFNSTYRVVSVLTVLHQDWLNGKEYKCKVSNKGLPSSIEKTISKAKGQPREPQVYTLPPSQEEMTKNQVSLTCLVKGFYPSDIAVEWESNGQPENNYKTTPPVLDSDGSFFLYSRLTVDKSRWQEGNVFSCSVMHEALHNHYTQKSLSLSLG

SEQ ID NO: 6 - protein, 214 aa, Homo sapiens
DIQMTQSPSSLSASVGDRVTITCHASQNINVWLSWYQQKPGKAPKLLIYKASNLHTGVPSRFTGSGSGTDFTFTISSLQPEDIATYYCQQGQTYPYTFGQGTKLEIKRTVAAPSVFIFPPSDEQLKSGTASVVCLLNNFYPREAKVQWKVDNALQSGNSQESVTEQDSKDSTYSLSSTLTLSKADYEKHKVYACEVTHQGLSSPVTKSFNRGEC

SEQ ID NO: 7 - protein, 214 aa, Homo sapiens
DIQMTQSPSSLSASVGDRVTITCHASQNINVWLSWYQQKPGKAPKLLIYKASNLHTGVPSRFSGSGSGTDFTFTISSLQPEDIATYYCQQGQTYPYTFGQGTKLEIKRTVAAPSVFIFPPSDEQLKSGTASVVCLLNNFYPREAKVQWKVDNALQSGNSQESVTEQDSKDSTYSLSSTLTLSKADYEKHKVYACEVTHQGLSSPVTKSFNRGEC

SEQ ID NO: 8 - DNA, 1356 bp, Homo sapiens
caggtccaactggtgcagtctggggctgaagtgaagaagcctggggcttcagtgaagttgtcctgcaaggcttctggctacatcttcaccagatactatatgtattgggtgaagcagaggcctggacaaggccttgagtggattggagagattaatcctaacaatggtggtactaagttcaatgagaagttcaagaacagggccacactgactgtagacaaatccatcagcacagcatacatggagctcagcaggctgagatctgacgacacggcggtctattattgttcaagagaggatgattacgacgggaccccctttgctatggactactggggtcaaggaaccctggtcaccgtctcctcagcctccaccaagggcccatcggtcttccccctggcaccctcctccaagagcacctctgggggcacagcggccctgggctgcctggtcaaggactacttccccgaaccggtgacggtgtcgtggaactcaggcgccctgaccagcggcgtgcacaccttcccggctgtcctacagtcctcaggactctactccctcagcagcgtggtgaccgtgccctccagcagcttgggcacccagacctacatctgcaacgtgaatcacaagcccagcaacaccaaggtggacaagagagttgagcccaaatcttgtgacaaaactcacacatgcccaccgtgcccagcacctgaattcgaggggggaccgtcagtcttcctcttccccccaaaacccaaggacaccctcatgatctcccggacccctgaggtcacatgcgtggtggtggacgtgagccacgaagaccctgaggtcaagttcaactggtacgtggacggcgtggaggtgcataatgccaagacaaagccgcgggaggagcagtacaacagcacgtaccgtgtggtcagcgtcctcaccgtcctgcaccaggactggctgaatggcaaggagtacaagtgcaaggtctccaacaaagccctcccagcctccatcgagaaaaccatctccaaagccaaagggcagccccgagaaccacaggtgtacaccctgcccccatcccgggaagagatgaccaagaaccaggtcagcctgacctgcctggtcaaaggcttctatcccagcgacatcgccgtggagtgggagagcaatgggcagccggagaacaactacaagaccacgcctcccgtgctggactccgacggctccttcttcctctatagcaagctcaccgtggacaagagcaggtggcagcaggggaacgtcttctcatgctccgtgatgcatgaggctctgcacaaccactacacgcagaagagcctctccctgtctccgggttga

SEQ ID NO: 9 - DNA, 1347 bp, Homo sapiens
caggtccaactggtgcagtctggggctgaagtgaagaagcctggggcttcagtgaagttgtcctgcaaggcttctggctacatcttcaccagatactatatgtattgggtgaagcagaggcctggacaaggccttgagtggattggagagattaatcctaacaatggtggtactaagttcaatgagaagttcaagaacagggccacactgactgtagacaaatccatcagcacagcatacatggagctcagcaggctgagatctgacgacacggcggtctattattgttcaagagaggatgattacgacgggaccccctttgctatggactactggggtcaaggaaccctggtcaccgtctcctcagcttccaccaagggcccatccgtcttccccctggcgccctgctccaggagcacctccgagagcacagccgccctgggctgcctggtcaaggactacttccccgaaccggtgacggtgtcgtggaactcaggcgccctgaccagcggcgtgcacaccttcccggctgtcctacagtcctcaggactctactccctcagcagcgtggtgaccgtgccctccagcagcttgggcacgaagacctacacctgcaatgtagatcacaagcccagcaacaccaaggtggacaagagagttgagtccaaatatggtcccccatgcccaccatgcccagcacctgagttcgaggggggaccatcagtcttcctgttccccccaaaacccaaggacactctcatgatctcccggacccctgaggtcacgtgcgtggtggtggacgtgagccaggaagaccccgaggtccagttcaactggtacgtggatggcgtggaggtgcataatgccaagacaaagccgcgggaggagcagttcaacagcacgtaccgtgtggtcagcgtcctcaccgtcctgcaccaggactggctgaacggcaaggagtacaagtgcaaggtctccaacaaaggcctcccgtcctccatcgagaaaaccatctccaaagccaaagggcagccccgagagccacaggtgtacaccctgcccccatcccaggaggagatgaccaagaaccaggtcagcctgacctgcctggtcaaaggcttctaccccagcgacatcgccgtggagtgggagagcaatgggcagccggagaacaactacaagaccacgcctcccgtgctggactccgacggctccttcttcctctacagcaggctaaccgtggacaagagcaggtggcaggaggggaatgtcttctcatgctccgtgatgcatgaggctctgcacaaccactacacacagaagagcctctccctgtctctgggttga

SEQ ID NO: 10 - DNA, 645 bp, Homo sapiens
gacatccagatgacccagtctccatccagtctgtctgcatccgtaggagacagagtcaccatcacttgccatgccagtcagaacattaatgtttggttatcttggtaccagcagaaaccaggaaaagcccctaaactcttgatctataaggcttccaacttgcacacaggcgtcccatcaagatttactggcagtggatctggaacagatttcacattcaccatcagcagcctgcagcctgaagacattgccacttactactgtcaacagggtcaaacttatccatacacgttcggacaggggaccaagctggagatcaaacgaactgtggctgcaccatctgtcttcatcttcccgccatctgatgagcagttgaaatctggaactgcctctgttgtgtgcctgctgaataacttctatcccagagaggccaaagtacagtggaaggtggataacgccctccaatcgggtaactcccaggagagtgtcacagagcaggacagcaaggacagcacctacagcctcagcagcaccctgacgctgagcaaagcagactacgagaaacacaaagtctacgcctgcgaagtcacccatcagggcctgagctcgcccgtcacaaagagcttcaacaggggagagtgttag

SEQ ID NO: 11 - DNA, 645 bp, Homo sapiens
gacatccagatgacccagtctccatccagtctgtctgcatccgtaggagacagagtcaccatcacttgccatgccagtcagaacattaatgtttggttatcttggtaccagcagaaaccaggaaaagcccctaaactcttgatctataaggcttccaacttgcacacaggcgtcccatcaagatttagtggcagtggatctggaacagatttcacattcaccatcagcagcctgcagcctgaagacattgccacttactactgtcaacagggtcaaacttatccatacacgttcggacaggggaccaagctggagatcaaacgaactgtggctgcaccatctgtcttcatcttcccgccatctgatgagcagttgaaatctggaactgcctctgttgtgtgcctgctgaataacttctatcccagagaggccaaagtacagtggaaggtggataacgccctccaatcgggtaactcccaggagagtgtcacagagcaggacagcaaggacagcacctacagcctcagcagcaccctgacgctgagcaaagcagactacgagaaacacaaagtctacgcctgcgaagtcacccatcagggcctgagctcgcccgtcacaaagagcttcaacaggggagagtgttag

SEQ ID NO: 12 - protein, 5 aa, Homo sapiens
RYYMY

SEQ ID NO: 13 - protein, 17 aa, Homo sapiens
EINPNNGGTKFNEKFKN

SEQ ID NO: 14 - protein, 13 aa, Homo sapiens
EDDYDGTPFAMDY

SEQ ID NO: 15 - protein, 11 aa, Homo sapiens
HASQNINVWLS

SEQ ID NO: 16 - protein, 7 aa, Homo sapiens
KASNLHT

SEQ ID NO: 17 - protein, 9 aa, Homo sapiens
QQGQTYPYT

SEQ ID NO: 18 - protein, 513 aa, Homo sapiens
MKMASFLAFLLLNFRVCLLLLQLLMPHSAQFSVLGPSGPILAMVGEDADLPCHLFPTMSAETMELKWVSSSLRQVVNVYADGKEVEDRQSAPYRGRTSILRDGITAGKAALRIHNVTASDSGKYLCYFQDGDFYEKALVELKVAALGSDLHVDVKGYKDGGIHLECRSTGWYPQPQIQWSNNKGENIPTVEAPVVADGVGLYAVAASVIMRGSSGEGVSCTIRSSLLGLEKTASISIADPFFRSAQRWIAALAGTLPVLLLLLGGAGYFLWQQQEEKKTQFRKKKREQELREMAWSTMKQEQSTRVKLLEELRWRSIQYASRGERHSAYNEWKKALFKPADVILDPKTANPILLVSEDQRSVQRAKEPQDLPDNPERFNWHYCVLGCESFISGRHYWEVEVGDRKEWHIGVCSKNVQRKGWVKMTPENGFWTMGLTDGNKYRTLTEPRTNLKLPKPPKKVGVFLDYETGDISFYNAVDGSHIHTFLDVSFSEALYPVFRILTLEPTALTICPA

SEQ ID NO: 19 - protein, 334 aa, Homo sapiens
MKMASSLAFLLLNFHVSLLLVQLLTPCSAQFSVLGPSGPILAMVGEDADLPCHLFPTMSAETMELKWVSSSLRQVVNVYADGKEVEDRQSAPYRGRTSILRDGITAGKAALRIHNVTASDSGKYLCYFQDGDFYEKALVELKVAALGSNLHVEVKGYEDGGIHLECRSTGWYPQPQIQWSNAKGENIPAVEAPVVADGVGLYEVAASVIMRGGSGEGVSCIIRNSLLGLEKTASISIADPFFRSAQPWIAALAGTLPILLLLLAGASYFLWRQQKEITALSSEIESEQEMKEMGYAATEREISLRESLQEELKRKKIQYLTRGEESSSDTNKSA

SEQ ID NO: 20 - protein, 584 aa, Homo sapiens
MKMASSLAFLLLNFHVSLFLVQLLTPCSAQFSVLGPSGPILAMVGEDADLPCHLFPTMSAETMELRWVSSSLRQVVNVYADGKEVEDRQSAPYRGRTSILRDGITAGKAALRIHNVTASDSGKYLCYFQDGDFYEKALVELKVAALGSDLHIEVKGYEDGGIHLECRSTGWYPQPQIKWSDTKGENIPAVEAPVVADGVGLYAVAASVIMRGSSGGGVSCIIRNSLLGLEKTASISIADPFFRSAQPWIAALAGTLPISLLLLAGASYFLWRQQKEKIALSRETEREREMKEMGYAATEQEISLREKLQEELKWRKIQYMARGEKSLAYHEWKMALFKPADVILDPDTANAILLVSEDQRSVQRAEEPRDLPDNPERFEWRYCVLGCENFTSGRHYWEVEVGDRKEWHIGVCSKNVERKKGWVKMTPENGYWTMGLTDGNKYRALTEPRTNLKLPEPPRKVGIFLDYETGEISFYNATDGSHIYTFPHASFSEPLYPVFRILTLEPTALTICPIPKEVESSPDPDLVPDHSLETPLTPGLANESGEPQAEVTSLLLPAHPGAEVSPSATTNQNHKLQARTEALY

SEQ ID NO: 21 - protein, 243 aa, Macaca fascicularis
MGSSLAFLLLSFHVCVLLLQLLMPHSAQFAVVGPPGPILAMVGEDADLPCHLFPTMSAETMELRWVSSNLRQVVNVYADGKEVEDRQSAAYRGRTSILRDGITAGKAALRIHNVTASDSGKYLCYFQDGDFYEKALVELKVAALGSDLHIDVKGYEDGGIHLECRSTGWYPQPQIRWSNDKGENIPAVEAPVFVDGVGLYAVAASVILRGSSGEGVSCTIRSSLLGLEKTTSISIAGHHHHHH

SEQ ID NO: 22 - protein, 243 aa, Macaca fascicularis
MGSSLAFLLLNFHVSFFLVQLLTPCSAQFSVLGPSGPILAMVGEDADLPCHLFPTMSAETMELRWVSSSLRQVVNVYADGKEVEDRQSAPYRGRTSILRDDIAAGKAALRIHNVTASDSGKYLCYFQDADFYEKALVELKVAALGSNLHVEVKGYEDGGIHLECRSTGWYPQPKIQWSNAKGQNIPAVEAPVVADGVGLYAVAASVIMRGGSGESVSCIIRNSVLGLEKTASISIADHHHHHH

SEQ ID NO: 23 - protein, 243 aa, Macaca fascicularis
MANFLAFLLLNFRVCLLLVQLLTPCSAQFAVLGPHGPILAMVGEDVDLPCHLFPTMSAETMELRWVSSSLRQVVNVYSDGKEVEDRQSAPYRGRTSILRDGITAGKAALRIHNVTASDSGKYLCYFQDGDFYEKALVELKVAALGSDLHIEVKGYEDGGIHLECRSTGWYPQPQIQWSNTKGQHIPAVKAPVVADGVGLYAVAASVIMRGSSGEGVSCIIRNSLLGLEKTASISITDHHHHHH